European Patent Application EP 4 647 500 A1, published November 12, 2025. Title: A process preparing L-glufosinate directly from L-homoserine. Applicant: 湖南利尔生物科技有限公司. The sequence listing filed with the application follows.

SEQUENCE LISTING (31 sequences)

SEQ ID NO: 1 - protein, 304 aa, Thermus thermophilus
MRVEGAIGKTPVVRLAKVVEPDMAEVWVKLEGLNPGGSIKDRPAWYMIKDAEERGILRPGSGQVIVEPTSGNTGIGLAMIAASRGYRLILTMPAQMSEERKRVLKAFGAELVLTDPERRMLAAREEALRLKEELGAFMPDQFKNPANVRAHYETTGPELYEALEGRIDAFVYGSGTGGTITGVGRYLKERIPHVKVIAVEPARSNVLSGGKMGQHGFQGMGPGFIPENLDLSLLDGVIQVWEEDAFPLARRLAREEGLFLGMSSGGIVWAALQVARELGPGKRVACISPDGGWKYLSTPLYAEP

SEQ ID NO: 2 - protein, 371 aa, Lysinibacillus sphaericus
MTLNRSIETKLVQLGNLSDPTTGAVSPPIHLSTAYKHAGIGESTGFDYTRTKNPTRALLEAGFADLEGGDMGFACSSGMAAIQLVLSIFKPGDELVVPDDLYGGTYRLFNFFQETYNIKPVYSKFESVEQVEALINEHTRALFIETPTNPLMQEFDLQVYAELAHKHGALLIVDNTFYTPYFQRPIDLGADIVLHSATKYIGGHNDVLAGIVVAKGTELAERIGFIHNGSGMVLGAMDSWLLIRGLKTMHLRLKQHDANAKAIAAYLEEEALVTDVLYTGKGGMLSFRLQKPEWIDPFLRNLKLITFAESLGGVESFITYPATQTHADMPYEERVERGVCDRLLRFSVGIEEAEDLIADLRQVFDILRKEA

SEQ ID NO: 3 - protein, 421 aa, Clostridioides difficile
MDNKETICVQGNYKPGNGEPRVLPLYQSTTFKYSSIDQLAELFDLKVDGHIYSRISNPTIQAFEEKISLLEGGVSSVAVSSGQSANMLAVLNICKSGDSILCSSKVYGGTFNLLGPSLKKFGIDLISFDLDSSEDEIVELAKENTKVVFAETLANPTLEVIDFEKIANVAKRINVPFIVDNSLASPVLCNPLKYGANIVTHSTTKYLDGHASSVGGIIVDGGNFNWDNGKFPELVEPDPTYHGISYTQKFGNAAYATKARVQLLRDYGNCLSPFNAYLTNLNVETLHLRMERHSENALKIARFLEKHENVDWINYPGLEDNKYYENAKKYLSRGCSGVLSFGVRGGLENAKKFVEKLQIASLVTHVSDVRTCVIHPASTTHRQLTEEQLIASGVLPSLIRLSVGIENVEDLIADLNQALNF

SEQ ID NO: 4 - protein, 425 aa, Clostridium novyi
MNNWKKGTICIQGGYTPKSGEPRVLPIYQSTTYKYNDPDEVAALFDLKAEGHMYSRISNPTVAAFEEKIAALEGGVGALAVASGQSASTLSILNVCKSGEHVVAASTLYGGTYSLFSTTLKKFGIDVTFVDPEATEEEILKNCRENTKAVFGETIGNPGLNVLDFEKFSNVAKKIKAPFIVDNTIATPYLCNPLKLGANVVVHSATKYIDGHATTVGGVIIDGGNFDWNNGRFPDFTEPDPSYHGIKYTETFGDSAYIVKARVQLLRDLGVCTSPFNAFLFSLGLETLHLRMERHSDNAIKLGRFLEKHSKVSWVSYPLLESHSTYETAKKYLPKGASGILTFGVKGGVEAGKQFIRNLKLAALVVHLGDARTSVLHPASTTHRQLTEEEQLSAGVTPDLIRVSVGIEDIEDIIEDFDQALNNIK

SEQ ID NO: 5 - protein, 434 aa, Geobacillus stearothermophilus
MSNEQTFRPETLAIHAGQKPDAETGARAVPIYQTSSYVFRDSEHAANLFGLKEEGFIYTRIMNPTNDVFEKRIAALEGGIGALALSSGQAAVFYSIINIASAGDEIVSSSSIYGGTYNLFAHTLRKFGITVKFVDPSDPENFERAITDKTKALFAETIGNPKNDVLDIEAVADIAHRHAIPLIVDNTVASPYLLRPIEFGADIVVHSATKFIGGHGNSIGGVIVDSGKFDWKGSGKFPEFTEPDPSYHGLVYVDAVGEAAYITKARIQLLRDLGAALSPFNAFLLLQGLETLHLRMQRHSENALAVAKFLEEEEAVESVNYPGLPSHPSHELAKKYLPNGQGAIVTFEIKGGVEAGKKLIDSVKLFSHLANIGDSKSLIIHPASTTHEQLSPDEQLSAGVTPGLVRLSVGTEAIDDILDDLRQAIRQSQTVGVK

SEQ ID NO: 6 - protein, 430 aa, Thermotoga maritima
MDWKKYGYNTRALHAGYEPPEQATGSRAVPIYQTTSYVFRDSDHAARLFALEEPGFIYTRIGNPTVSVLEERIAALEEGVGALAVASGQAAITYAILNIAGPGDEIVSGSALYGGTYNLFRHTLYKKSGIIVKFVDETDPKNIEEAITEKTKAVYLETIGNPGLTVPDFEAIAEIAHRHGVPLIVDNTVAPYIFRPFEHGADIVVYSATKFIGGHGTSIGGLIVDSGKFDWTNGKFPELVEPDPSYHGVSYVETFKEAAYIAKCRTQLLRDLGSCMSPFNAFLFILGLETLSLRMKKHCENALKIVEFLKSHPAVSWVNYPIAEGNKTRENALKYLKEGYGAIVTFGVKGGKEAGKKFIDSLTLISHLANIGDARTLAIHPASTTHQQLTEEEQLKTGVTPDMIRLSVGIEDVEDIIADLDQALRKSQEG

SEQ ID NO: 7 - protein, 425 aa, Pseudomonas aeruginosa
MKLETLAVHAGYSPDPTTRAVAVPIYQTTSYAFDDTQHGADLFDLKVPGNIYTRIMNPTNDVLEQRVAALEGGVGALAVASGMAAITYAIQTVAEAGDNIVSVAKLYGGTYNLLAHTLPRIGIQARFAAHDDVAALEALIDERTKAVFCETIGNPAGNIIDLQALADAAHRHGVPLIVDNTVATPVLCRPFEHGADIVVHSLTKYMGGHGTSIGGIVVDSGKFDWAANKSRFPLLNTPDPSYHGVTYTEAFGPAAFIGRCRVVPLRNMGAALSPFNAFLILQGLETLALRMERHCDNALAVARYLQQHPQVAWVKYAGLADNPEHALARRYLGGRPAAILSFGIQGGSAAGARFIDALKLVVRLVNIGDAKSLACHPASTTHRQLNAEELARAGVSDDMVRLSIGIEHIDDILADLDQALAAAAR

SEQ ID NO: 8 - protein, 346 aa, Nonlabens dokdonensis
MSNNIKAYNNVLELIGETPLIKLSQTVASFPGNYYAKAEAFNPGHSSKDRIALHIIEQAEKKGILKPGDTIIETTSGNTGFSIAMVSRIKGYDCILAVSSKSSADKIDMLKSMGAKVYVCPANVSADDPRSYYQVAKRLHDEIKNSIYINQYFNDLNTEAHYLTTGPEIWNQTAGEITHLVACSGTGGTISGTARFLKEQNPNIKILGVDAYGSVLKKYHETQEFDKDEIYPYRIEGLGKNLIPTATDFDVIDSFTKVKDEDAAHMARKISQTEGLFVGYTSGAAMQAVKQLVVEGEFDKNSNVVVIFPDHGSRYMSKIYNDQWMQEQGFVDSKSTANEQHIEYIK

SEQ ID NO: 9 - protein, 325 aa, Leucaena leucocephala
MAVEWTGIANDVTELVGKTPLVYLNKVVDGCVGRIVAKLEFMEPLSSVKDRIGYSMIADAEEKGLITPGKSVLIEPTSGNTGIGLAFTAAAKGYRLIIVMPASMTLERRMVLKALGAELVLTDPEKGIRGAFQKVEEIYAKTPNSYVLQQFENPSNPKMHYDTTGPEIWKATGGKIDALVAGIGTGGTITGSGKFLKEQNPNIKVCAVEPAESPVLVGGQPGSHGIYGIGAGFIPKVVDVSLLDEVVHVTTSEAIETAKLLAVKEGLFVGVSSGAAAAAAIKVAKRPEMAGKLIVTIFPSCGERYLSSALFESIREESENMTFEP

SEQ ID NO: 10 - protein, 308 aa, Aeropyrum pernix
MVFPSPLDFFERGKPTPLVRSRLQLPNGVRVWLKLEWYNPFSLSVKDRPAVEIISRLSRRVEKGSLVADATSSNFGVALSAVARLYGYRARVYLPGAAEEFGKLLPRLLGAQVIVDPEAPSTVHLLPRVMKDSKNEGFVHVNQFYNDANFEAHMRGTAREIFVQSRRGGLALRGVAGSLGTSGHMSAAAFYLQSVDPSIRAVLVQPAQGDSIPGIRRVETGMLWINMLDISYTLAEVTLEEAMEAVVEVARSDGLVIGPSGGAAVKALAKKAAEGDLEPGDYVVVVPDTGFKYLSLVQNALEGAGDSV

SEQ ID NO: 11 - protein, 416 aa, Methanosarcina acetivorans
MGRFILKCLKCGREYSQEYRLTCENDDSFLRAEYLEKKLELRKQPGIGRFHSWLPVQEELTTEAGPITYKSEALARELGLSNLYIGFSGYWPEKGAFIKTCSFKELEAHPTMQLLKESGGKAIVLASAGNTGRAFAHVSALTGTDVYIVVPDSGIPKLWLPEEPTDSIHLISMTPGNDYTDAINLAGRIAKLPGMVPEGGARNVARREGMGTVMLDAAVTIGKMPDHYFQAVGSGTGGISAWEASLRLREDGRFGSKLPKLQLTQNLPFVPMYNAWQEGRRDIIPEIDMKDAKKRIEETYATVLTNRAPPYSVTGGLYDALVDTDGIMYAVSKEEALDAKALFESLEGIDILPPSAVAAASLLKAVEAGNVGKDDTILLNIAGGGFKRLKEDFTLFQIEPEITVSNPDVPLEELKL

SEQ ID NO: 12 - protein, 323 aa, Mycobacterium tuberculosis
MTRYDSLLQALGNTPLVGLQRLSPRWDDGRDGPHVRLWAKLEDRNPTGSIKDRPAVRMIEQAEADGLLRPGATILEPTSGNTGISLAMAARLKGYRLICVMPENTSVERRQLLELYGAQIIFSAAEGGSNTAVATAKELAATNPSWVMLYQYGNPANTDSHYCGTGPELLADLPEITHFVAGLGTTGTLMGTGRFLREHVANVKIVAAEPRYGEGVYALRNMDEGFVPELYDPEILTARYSVGAVDAVRRTRELVHTEGIFAGISTGAVLHAALGVGAGALAAGERADIALVVADAGWKYLSTGAYAGSLDDAETALEGQLWA

SEQ ID NO: 13 - protein, 307 aa, Bacillus subtilis
MTVITDITELIGNTPLLRLKNFDVPEGVAVYAKLEMMNPGGSIKDRLGDMLIRDALDSGKVKPGGVIIEATAGNTGIGLALSARKYGLKAIFCVPEHFSREKQQIMQALGASIIHTPRQDGMQGAIQKAIQLETEIENSYCVLQFKNRVNPSTYYKTLGPEMWEALDGNIHTFVAGAGSGGTFAGTASFLKEKNPAVKTVIVEPVGSILNGGEPHAHKTEGIGMEFIPDYMDKSHFDEIYTVTDENAFRLVKEAAEKEGLLIGSSSGAALYAALEEAKKASAGTNIVTVFPDSSDRYISKQIYEGGI

SEQ ID NO: 14 - protein, 306 aa, Staphylococcus aureus
MVQLHQLFPKHEVFAKLEYMNPGGSMKDRPAKYIIEHGIKHGLITENTHLIESTSGNLGIALAMIAKIKGLKLTCVVDPKISPTNLKIIKSYGANVEMVEEPDAHGGYLMTRIAKVQELLATIDDAYWINQYANELNWQSHYHGAGTEIVETIKQPIDYFVAPVSTTGSIMGMSRKIKEVHPNAQIVAVDAKGSVIFGDKPINRELPGIGASRVPEILNRSEINQVIHVDDYQSALGCRKLIDYEGIFAGGSTGSIIAAIEQLITSIEEGATIVTILPDRGDRYLDLVYSDTWLEKMKSRQGVKSE

SEQ ID NO: 15 - protein, 300 aa, Pseudomonas fluorescens
MTLQYPTIADCVGNTPLVRLQRMAGNTSNTLLLKLEGNNPAGSVKDRPALSMITRAELRGQIKPGDTLIEATSGNTGIALAMAAAIKGYKMILIMPDNGSAERKAAMTAYGAELLLVTPEEGMEGARDLAERMAAEGRGQVLDQFANGDNPEAHYTSTGPEIWRQTQGTITHFVSSMGTTGTIMGNSRYLKEQNPAIQIVGLQPMEGAAIPGIRRWPQEYLPKIYNAARVDRIIDMAQREAEDTTRRLAREEGIFCGVSSGGAVAGMLRLSAELENAVIVAIICDRGDRYLSTGIFDAPN

SEQ ID NO: 16 - protein, 398 aa, Escherichia coli
MSVFSLKIDIADNKFFNGETSPLFSQSQAKLARQFHQKIAGYRPTPLCALDDLANLFGVKKILVKDESKRFGLNAFKMLGGAYAIAQLLCEKYHLDIETLSFEHLKNAIGEKMTFATTTDGNHGRGVAWAAQQLGQNAVIYMPKGSAQERVDAILNLGAECIVTDMNYDDTVRLTMQHAQQHGWEVVQDTAWEGYTKIPTWIMQGYATLADEAVEQMREMGVTPTHVLLQAGVGAMAGGVLGYLVDVYSPQNLHSIIVEPDKADCIYRSGVKGDIVNVGGDMATIMAGLACGEPNPLGWEILRNCATQFISCQDSVAALGMRVLGNPYGNDPRIISGESGAVGLGVLAAVHYHPQRQSLMEKLALNKDAVVLVISTEGDTDVKHYREVVWEGKHAVAP

SEQ ID NO: 17 - protein, 454 aa, Escherichia coli
MISAFDIFKIGIGPSSSHTVGPMNAGKSFIDRLESSGLLTATSHIVVDLYGSLSLTGKGHATDVAIIMGLAGNSPQDVVIDEIPAFIELVTRSGRLPVASGAHIVDFPVAKNIIFHPEMLPRHENGMRITAWKGQEELLSKTYYSVGGGFIVEEEHFGLSHDVETSVPYDFHSAGELLKMCDYNGLSISGLMMHNELALRSKAEIDAGFARIWQVMHDGIERGMNTEGVLPGPLNVPRRAVALRRQLVSSDNISNDPMNVIDWINMYALAVSEENAAGGRVVTAPTNGACGIIPAVLAYYDKFRRPVNERSIARYFLAAGAIGALYKMNASISGAEVGCQGEIGVACSMAAAGLTELLGGSPAQVCNAAEIAMEHNLGLTCDPVAGQVQIPCIERNAINAVKAVNAARMAMRRTSAPRVSLDKVIETMYETGKDMNDKYRETSRGGLAIKVVCG

SEQ ID NO: 18 - protein, 442 aa, Escherichia coli
MENAKMNSLIAQYPLVKDLVALKETTWFNPGTTSLAEGLPYVGLTEQDVQDAHARLSRFAPYLAKAFPETAATGGIIESELVAIPAMQKRLEKEYQQPISGQLLLKKDSHLPISGSIKARGGIYEVLAHAEKLALEAGLLTLDDDYSKLLSPEFKQFFSQYSIAVGSTGNLGLSIGIMSARIGFKVTVHMSADARAWKKAKLRSHGVTVVEYEQDYGVAVEEGRKAAQSDPNCFFIDDENSRTLFLGYSVAGQRLKAQFAQQGRIVDADNPLFVYLPCGVGGGPGGVAFGLKLAFGDHVHCFFAEPTHSPCMLLGVHTGLHDQISVQDIGIDNLTAADGLAVGRASGFVGRAMERLLDGFYTLSDQTMYDMLGWLAQEEGIRLEPSALAGMAGPQRVCASVSYQQMHGFSAEQLRNTTHLVWATGGGMVPEEEMNQYLAKGR

SEQ ID NO: 19 - protein, 502 aa, Candida maltosa
MSIVRLYTARQLPRYRPLRFVRFNSTQVLSPKQRWTELKDTDFIKDSNGEEQPDYVKLILTSRVYDVVDDAGSPLTYAINLSHRCGTNVYLKREDLLPVFSFKLRGAYNMIAHLHSNSPTPVPGVIACSAGNHAQGVAFSANKLNIPATIVMPTPTPSIKYTNVSRLGSQVVLYGDDFDSAKQECARLSAEQNLIDIPPFNHPYVIAGQGTVALEITRQLRLDKLDAIFVPVGGGGLIAGIAVYLKQIAPHVKIIGVETYDADAMYQSLKNHKSTVLDKVGLFADGTAVKVLGDETWRLAKDLVDEVVLVTTDELCAAIKDIFEDTRSITEPSGALSVAGLKRYIEDHSEIDHKGKTYVPVLSGANMNFDRLRFVSERAVLGEGREVSLAVTIPEQPGEFAKLQKLINPRAITEFSYRTSGEPTANIFVSFNVIDKKKEKALVINAMTEAGYKVVDISENELAKSHGRYLVGGKSSIMVMILVKSCVDSISQKDSKKNSNNS

SEQ ID NO: 20 - protein, 384 aa, Streptomyces phaeochromogenes
MTDSVTGAGDGTRAVRAGLPEPVKHEPTLPGPVFAAHFHLPGDPTGPYTYGRDENPTWTHLERAIGELEAPGRDDVETLVFASGMAAISAVLFSQLSAGDTVVLPDDGYQVLPLVRAQLEAYGVEVRTAPTGGDAQLDVLDGAKLLWIETPSNPGLDVCDVRRLVEAAHARGCLVAVDNTLATPLGQRPLELGADFSVASGTKQLTGHGDILLGYVTGGDAAAMASVRRWRKIVGAIPGPMEAWLAHRSIATLQLRVDRQNANALVIAEALRDRHEDLGVRYPGLPGDPSHKIASQQMRRFGCVVSFTLPTRARADRFLDALRLVDDATSFGGVRSTAERRGRWGGDAVPEGFIRFSAGAEDPQDLVADVLRALNESSQPTPSE

SEQ ID NO: 21 - protein, 417 aa, Neurospora crassa
MTASSDHPITTPPRAPSPVHGFGTLAVHAGSPHDPATGAVIEAISLSTTFAQTAVGKPVGEFEYSRSSNPNRANFEKMVAALEHAKYALAYSSGSATTANILQSLAAGSHVISVSDVYGGTHRYFTQVAKAHGVKVTFTPEIEVDIRDHITDATKLVWIETPSNPTLRLVDIRAVATAAHERGILVVVDNTFLSPYVQNPLDHGADIVVHSVTKYINGHSDVVMGVAAFNSDELYARLSFLQNAIGAVPSAFDSWLAHRGAKTLHLRAREATTNATAIAHALEASPLVISVNYPGLESHPHRAIALKQHRNGMGGGMLSFRIHGGHAAAEKFCQYTKIFTLAESLGGVESLCEIPSSMTHAGIPKAQREAVGIFDDLVRISCGVEDAEDLKADVLQALERAVADAANGVSNGVNGTH

SEQ ID NO: 22 - protein, 379 aa, Bacillus subtilis
MKKKTLMIHGGITGDEKTGAVSVPIYQVSTYKQPKAGQHTGYEYSRTANPTRTALEALVTELESGEAGYAFSSGMAAITAVMMLFNSGDHVVLTDDVYGGTYRVMTKVLNRLGIESTFVDTSSREEVEKAIRPNTKAIYIETPTNPLLKITDLTLMADIAKKAGVLLIVDNTFNTPYFQQPLTLGADIVLHSATKYLGGHSDVVGGLVVTASKELGEELHFVQNSTGGVLGPQDSWLLMRGIKTLGLRMEAIDQNARKIASFLENHPAVQTLYYPGSSNHPGHELAKTQGAGFGGMISFDIGSEERVDAFLGNLKLFTIAESLGAVESLISVPARMTHASIPRERRLELGITDGLIRISVGIEDAEDLLEDIGQALENI

SEQ ID NO: 23 - protein, 368 aa, Spinacia oleracea
MATVSSCLLRRSRTASRIFKTSLRCFSTTSSSAQTVSGSSPFPFTGTNIKTNVSQLIGRTPLVYLSKISEGSGAYIAVKQEMMQPTASVKDRPALAMIEDAEKKGLISPGKTVLIEPTSGNMGISMAFMAAMKGYKMVLTMPSYTSMERRVVMRAFGADLILTDPDKGMGGTVKKANQLLDSTPDGFMLQQFNNPANTQVHFETTGPEIWEDTQGKVDIFVMGIGSGGTVSGVGRYLKSQNPNVKIYGVEPAESNILNGGKPGPHLITGNGVGFKPEILDMDVMDAVLEVKSDDAVKMARQLALQEGLLVGISSGANTIAALDLAKRPENKGKLIVTIHPSFGERYLSSALFKELREEAENMQPVPVE

SEQ ID NO: 24 - protein, 400 aa, Cyanobacteria bacterium
MSGIYPAPVRLESHRQQFPALANKAYFNYGGQGTLPQASLEAIQQAYEYIQRHGPFSAGVNAWIIEEANKTREAIASELGAPPEAIAITEDVTVGCNIAMWGINWQAGDHLLLTDCEHPSVIATAQEIARRFDVEVSTCPILSTLNQGDPTAVIAQHLRTQTRLVVLSHILWNTGQVLPVKEIVEVCRNYSSSSQTIRVLVDAAQSVGCLPLNLTELGADFYAFTGHKWWCGPEGIGGLYVRPDAWESLNPTFIGWRGIVSNQAGKPTGWKPNAQRFEVATSAYPLYAGVRSAIATHQQWGTPQERYQQICQISEYLWQRLSQLDFVKCLRTSPPQAGLVSFVLTNEHSHQQLVKSLEQQNLMLRTILDPNCVRACVHYFTQHAEIDKLIEAMKKIKSKG

SEQ ID NO: 25 - protein, 398 aa, Pseudomonas putida
MRDSHHNTGFSTRAIHHGYDPLSHGGALVPPVYQTATYAFPTVEYGAACFAGEEPGHFYSRISNPTLALLEQRMASLEGGEAGLALASGMGAITSTLWTLLRPGDELIVGRTLYGCTFAFLHHGIGEFGVKVRHVDLNDAKALKAAISSKTRMIYFETPANPNMQLVDIAAVVEAVRGHDVHVVVDNTYCTPYLQRPLELGADLVVHSATKYLSGHGDITAGLVVGRKVLVDRIRLEGLKDMTGAVLSPHDAALLMRGIKTLALRMDRHCANAQQVAEFLVRQPQVELIHYPGLPSFAQYALAQRQMRLPGGMIAFELKGGIEAGRRFMNALQLFARAVSLGDAESLAQHPASMTHSSYTPQERAHHGISEGLVRLSVGLEDVEDLLADVEQALQACC

SEQ ID NO: 26 - protein, 380 aa, Lactococcus lactis
MTSLKTKVIHGGISTDRTTGAVSVPIYQTSTYKQNGLGKPKEYEYSRSGNPTRHALEELIADLEGGVQGFAFSSGLAGIHAVLSLFSAGDHIILADDVYGGTFRLMDKVLTKTGIIYDLVDLSNLEDLKAAFKAETKAVYFETPSNPLLKVLDIKEISSIAKAHNALTLVDNTFATPYLQQPIALGADIVLHSATKYLGGHSDVVAGLVTTNSNELASEIGFLQNSIGAVLGPQDSWLVQRGIKTLALRMEAHSANAQKIAEFLEASQAVSKVYYPGLVNHEGHEIAKKQMTAFGGMISFELTDENAVKNFVENLRYFTLAESLGGVESLIEVPAVMTHASIPKELREEIGIKDGLIRLSVGVEALEDLLTDLKEALEKE

SEQ ID NO: 27 - protein, 328 aa, Escherichia coli
MPLHNLTRFPRLEFIGAPTPLEYLPRFSDYLGREIFIKRDDVTPMAMGGNKLRKLEFLAADALREGADTLITAGAIQSNHVRQTAAVAAKLGLHCVALLENPIGTTAENYLTNGNRLLLDLFNTQIEMCDALTDPNAQLEELATRVEAQGFRPYVIPVGGSNALGALGYVESALEIAQQCEGAVNISSVVVASGSAGTHAGLAVGLEHLMPESELIGVTVSRSVADQLPKVVNLQQAIAKELELTASAEILLWDDYFAPGYGVPNDEGMEAVKLLARLEGILLDPVYTGKAMAGLIDGISQKRFKDEGPILFIHTGGAPALFAYHPHV

SEQ ID NO: 28 - protein, 406 aa, Escherichia coli
MIFSVDKVRADFPVLSREVNGLPLAYLDSAASAQKPSQVIDAEAEFYRHGYAAVHRGIHTLSAQATEKMENVRKRASLFINARSAEELVFVRGTTEGINLVANSWGNSNVRAGDNIIISQMEHHANIVPWQMLCARVGAELRVIPLNPDGTLQLETLPTLFDEKTRLLAITHVSNVLGTENPLAEMITLAHQHGAKVLVDGAQAVMHHPVDVQALDCDFYVFSGHKLYGPTGIGILYVKEALLQEMPPWEGGGSMIATVSLSEGTTWTKAPWRFEAGTPNTGGIIGLGAALEYVSALGLNNIAEYEQNLMHYALSQLESVPDLTLYGPQNRLGVIAFNLGKHHAYDVGSFLDNYGIAVRTGHHCAMPLMAYYNVPAMCRASLAMYNTHEEVDRLVTGLQRIHRLLG

SEQ ID NO: 29 - protein, 339 aa, Ruegeria pomeroyi
MHLARYPRRFIAHLPTPLERLDRLTAELGGPEIWIKRDDCTGLSTGGNKTRKLEFLMAEAELQGADMVMTQGATQSNHARQTAAFAAKLGMDCHILLEDRTGSNNANYNNNGNVLLDHLHGATTEKRPGSGLDMNAEMEKVAEKFRADGRKVYTIPGGGSNPTGALGYVNCAFEMLNQFNERGLKVDHIVHATGSAGTQAGLITGLQAMNAQIPLLGIGVRAPKPKQEENVYNLACATAEKLGCPGVVAREDVVANTDYVGEGYGIPTESGLEAIRMFAELEAILLDPVYSAKGAAGFIDLIRKGHFKKGERVVFLHTGGAVALFGYDNAFDYSGRWVA

SEQ ID NO: 30 - protein, 396 aa, Methanococcus maripaludis
MDDYKRILITKILKNEVTEALGCTEVGLIGYAVSLCNISDPFSIEKIELTLNNGSFKNAYAVGVPNTKKYGILPAVVGGLLGDHKNKLLVFNGIKYSQKLEDFIKERLKIRVINSPLYCGVKIKDNSGNTFESLIKDNHLNVVIPKINNKLISEINGSEKEEYKNLELLDFLEYIDEIPEEIIQLVEKTIYTNNNLIKGDFLNFGNDCLSNMVNKTTSACNTRMIGENMPAMSVAKSGNMGIMATLPIIAYDYSNEQNQEKLIKSILLSVLVTIYATYKSSYLSSMCGCVSKGGMGAVIGLCYYKNGKNIKKLDSAARTFTANLPGIICDGGKVGCALKLASGCFAAYSSLFVDISYENGIVGKNFKECVENISEISKIMGDLDSDIVKIMSKKEI

SEQ ID NO: 31 - protein, 423 aa, Camelina sativa
MANDRSVDWKFSGSEAAKEASAASLGTYSSKLFALCDPLGKPILPPRSKSAETSHTAEKAVVEAVLCGTGNAYAPSLGLPVARSAVAEYLNRDLPKKLTADDVFMTVGGKQAIELTVDILAKPKANVLLPKPGFPWDVVRTIYKNLEVRKYDFIPEQNYEIDFDSVRALVDENTFAIFIINPHNPNGNTYSEVHLKKLAELARELRIMVVSDEVFRWTVFGSNPFVPMGKFSSIVPVVTLGSISKGWIVPGWRTGWVALHDLDGVFKCTKVLTAAKQFLVINSKPPTVIQAALPTILENTPEEFFHKRQKFLKEKADFAYSKLKEIPTLTCYLKPEACTFLWTELNLSRFADIKDDEEFCEKLATEENLVLLPGIAFGLKNWARHSIDMEISTLEDALGRLKSFCERHSIIIEVPLKDVNGVK